European Patent Application EP 4 722 364 A1, published April 8, 2026. Title: 一种抑制C5基因表达的dsRNA分子及其应用. Applicant: 石药集团中奇制药技术（石家庄）有限公司. Application CN. The sequence listing filed with the application follows.

SEQUENCE LISTING (212 sequences)

SEQ ID NO: 1 - RNA, 21 nt, Synthetic construct
  source 1..21: mol_type = other RNA
atttcagcaccaaaaatattc

SEQ ID NO: 2 - RNA, 21 nt, Synthetic construct
  source 1..21: mol_type = other RNA
ttcagcaccaaaaatattccg

SEQ ID NO: 3 - RNA, 21 nt, Synthetic construct
  source 1..21: mol_type = other RNA
tcagcaccaaaaatattccgt

SEQ ID NO: 4 - RNA, 21 nt, Synthetic construct
  source 1..21: mol_type = other RNA
tattgtgattcaagtttatgg

SEQ ID NO: 5 - RNA, 21 nt, Synthetic construct
  source 1..21: mol_type = other RNA
gtgattcaagtttatggatac

SEQ ID NO: 6 - RNA, 21 nt, Synthetic construct
  source 1..21: mol_type = other RNA
gattcaagtttatggatacac

SEQ ID NO: 7 - RNA, 21 nt, Synthetic construct
  source 1..21: mol_type = other RNA
agcatttgatgcaacaatctc

SEQ ID NO: 8 - RNA, 21 nt, Synthetic construct
  source 1..21: mol_type = other RNA
gcaacaatctctattaaaagt

SEQ ID NO: 9 - RNA, 21 nt, Synthetic construct
  source 1..21: mol_type = other RNA
caacaatctctattaaaagtt

SEQ ID NO: 10 - RNA, 21 nt, Synthetic construct
  source 1..21: mol_type = other RNA
tctctattaaaagttatcctg

SEQ ID NO: 11 - RNA, 21 nt, Synthetic construct
  source 1..21: mol_type = other RNA
agttatcctgataaaaaattt

SEQ ID NO: 12 - RNA, 21 nt, Synthetic construct
  source 1..21: mol_type = other RNA
atttatcctcagagaataaat

SEQ ID NO: 13 - RNA, 21 nt, Synthetic construct
  source 1..21: mol_type = other RNA
ttatcctcagagaataaattc

SEQ ID NO: 14 - RNA, 21 nt, Synthetic construct
  source 1..21: mol_type = other RNA
gagaataaattccaaaactct

SEQ ID NO: 15 - RNA, 21 nt, Synthetic construct
  source 1..21: mol_type = other RNA
tcttaacaatacaaccaaaac

SEQ ID NO: 16 - RNA, 21 nt, Synthetic construct
  source 1..21: mol_type = other RNA
cccagtttcttatgtgtattt

SEQ ID NO: 17 - RNA, 21 nt, Synthetic construct
  source 1..21: mol_type = other RNA
tgtgtatttggaagttgtatc

SEQ ID NO: 18 - RNA, 21 nt, Synthetic construct
  source 1..21: mol_type = other RNA
agttgtatcaaagcatttttc

SEQ ID NO: 19 - RNA, 21 nt, Synthetic construct
  source 1..21: mol_type = other RNA
cttcattcatacagacaaacc

SEQ ID NO: 20 - RNA, 21 nt, Synthetic construct
  source 1..21: mol_type = other RNA
acagacaaacctgtttatact

SEQ ID NO: 21 - RNA, 21 nt, Synthetic construct
  source 1..21: mol_type = other RNA
cagacaaacctgtttatactc

SEQ ID NO: 22 - RNA, 21 nt, Synthetic construct
  source 1..21: mol_type = other RNA
aacctgtttatactccagacc

SEQ ID NO: 23 - RNA, 21 nt, Synthetic construct
  source 1..21: mol_type = other RNA
agagtttattcgttgaatgac

SEQ ID NO: 24 - RNA, 21 nt, Synthetic construct
  source 1..21: mol_type = other RNA
ctgtcttaactttcatagatc

SEQ ID NO: 25 - RNA, 21 nt, Synthetic construct
  source 1..21: mol_type = other RNA
gtcttaactttcatagatcct

SEQ ID NO: 26 - RNA, 21 nt, Synthetic construct
  source 1..21: mol_type = other RNA
ttgatcatattggaattatct

SEQ ID NO: 27 - RNA, 21 nt, Synthetic construct
  source 1..21: mol_type = other RNA
tgatcatattggaattatctc

SEQ ID NO: 28 - RNA, 21 nt, Synthetic construct
  source 1..21: mol_type = other RNA
tcatattggaattatctcttt

SEQ ID NO: 29 - RNA, 21 nt, Synthetic construct
  source 1..21: mol_type = other RNA
ttttcctgacttcaagattcc

SEQ ID NO: 30 - RNA, 21 nt, Synthetic construct
  source 1..21: mol_type = other RNA
acttcaagattccgtctaatc

SEQ ID NO: 31 - RNA, 21 nt, Synthetic construct
  source 1..21: mol_type = other RNA
cttcaagattccgtctaatcc

SEQ ID NO: 32 - RNA, 21 nt, Synthetic construct
  source 1..21: mol_type = other RNA
ttccgtctaatcctagatatg

SEQ ID NO: 33 - RNA, 21 nt, Synthetic construct
  source 1..21: mol_type = other RNA
taatcctagatatggtatgtg

SEQ ID NO: 34 - RNA, 21 nt, Synthetic construct
  source 1..21: mol_type = other RNA
taaatataaagaggacttttc

SEQ ID NO: 35 - RNA, 21 nt, Synthetic construct
  source 1..21: mol_type = other RNA
attactataaaagcaagatat

SEQ ID NO: 36 - RNA, 21 nt, Synthetic construct
  source 1..21: mol_type = other RNA
aagcaagatatttttataata

SEQ ID NO: 37 - RNA, 21 nt, Synthetic construct
  source 1..21: mol_type = other RNA
ttttataataaagtagtcact

SEQ ID NO: 38 - RNA, 21 nt, Synthetic construct
  source 1..21: mol_type = other RNA
cactgaggctgacgtttatat

SEQ ID NO: 39 - RNA, 21 nt, Synthetic construct
  source 1..21: mol_type = other RNA
actgaggctgacgtttatatc

SEQ ID NO: 40 - RNA, 21 nt, Synthetic construct
  source 1..21: mol_type = other RNA
aaagatgatcaaaaagaaatg

SEQ ID NO: 41 - RNA, 21 nt, Synthetic construct
  source 1..21: mol_type = other RNA
aaaacacaatgttgataaatg

SEQ ID NO: 42 - RNA, 21 nt, Synthetic construct
  source 1..21: mol_type = other RNA
aaacacaatgttgataaatgg

SEQ ID NO: 43 - RNA, 21 nt, Synthetic construct
  source 1..21: mol_type = other RNA
tgtcatactacagtttagaag

SEQ ID NO: 44 - RNA, 21 nt, Synthetic construct
  source 1..21: mol_type = other RNA
aagatttaaacaacaagtacc

SEQ ID NO: 45 - RNA, 21 nt, Synthetic construct
  source 1..21: mol_type = other RNA
gatttaaacaacaagtacctt

SEQ ID NO: 46 - RNA, 21 nt, Synthetic construct
  source 1..21: mol_type = other RNA
aaacaacaagtacctttatat

SEQ ID NO: 47 - RNA, 21 nt, Synthetic construct
  source 1..21: mol_type = other RNA
aacaacaagtacctttatatt

SEQ ID NO: 48 - RNA, 21 nt, Synthetic construct
  source 1..21: mol_type = other RNA
acaacaagtacctttatattg

SEQ ID NO: 49 - RNA, 21 nt, Synthetic construct
  source 1..21: mol_type = other RNA
caacaagtacctttatattgc

SEQ ID NO: 50 - RNA, 21 nt, Synthetic construct
  source 1..21: mol_type = other RNA
ctttatattgctgtaacagtc

SEQ ID NO: 51 - RNA, 21 nt, Synthetic construct
  source 1..21: mol_type = other RNA
cagaaatacctggcatcaaat

SEQ ID NO: 52 - RNA, 21 nt, Synthetic construct
  source 1..21: mol_type = other RNA
caggttaaagattcgcttgac

SEQ ID NO: 53 - RNA, 21 nt, Synthetic construct
  source 1..21: mol_type = other RNA
aggttaaagattcgcttgacc

SEQ ID NO: 54 - RNA, 21 nt, Synthetic construct
  source 1..21: mol_type = other RNA
acggtgctggagtttaatgtc

SEQ ID NO: 55 - RNA, 21 nt, Synthetic construct
  source 1..21: mol_type = other RNA
ctggagtttaatgtcaaaact

SEQ ID NO: 56 - RNA, 21 nt, Synthetic construct
  source 1..21: mol_type = other RNA
tggagtttaatgtcaaaactg

SEQ ID NO: 57 - RNA, 21 nt, Synthetic construct
  source 1..21: mol_type = other RNA
gggaaggttaccgagcaatag

SEQ ID NO: 58 - RNA, 21 nt, Synthetic construct
  source 1..21: mol_type = other RNA
ggaaggttaccgagcaatagc

SEQ ID NO: 59 - RNA, 21 nt, Synthetic construct
  source 1..21: mol_type = other RNA
ccgagcaatagcatactcatc

SEQ ID NO: 60 - RNA, 21 nt, Synthetic construct
  source 1..21: mol_type = other RNA
atattgattggactgataacc

SEQ ID NO: 61 - RNA, 21 nt, Synthetic construct
  source 1..21: mol_type = other RNA
attattgttacccccaaaagc

SEQ ID NO: 62 - RNA, 21 nt, Synthetic construct
  source 1..21: mol_type = other RNA
cccaaaagcccatatattgac

SEQ ID NO: 63 - RNA, 21 nt, Synthetic construct
  source 1..21: mol_type = other RNA
ccatatattgacaaaataact

SEQ ID NO: 64 - RNA, 21 nt, Synthetic construct
  source 1..21: mol_type = other RNA
catatattgacaaaataactc

SEQ ID NO: 65 - RNA, 21 nt, Synthetic construct
  source 1..21: mol_type = other RNA
gacaaaataactcactataat

SEQ ID NO: 66 - RNA, 21 nt, Synthetic construct
  source 1..21: mol_type = other RNA
acaaaataactcactataatt

SEQ ID NO: 67 - RNA, 21 nt, Synthetic construct
  source 1..21: mol_type = other RNA
caaaataactcactataatta

SEQ ID NO: 68 - RNA, 21 nt, Synthetic construct
  source 1..21: mol_type = other RNA
aactcactataattacttgat

SEQ ID NO: 69 - RNA, 21 nt, Synthetic construct
  source 1..21: mol_type = other RNA
tttatccaagggcaaaattat

SEQ ID NO: 70 - RNA, 21 nt, Synthetic construct
  source 1..21: mol_type = other RNA
ttatccaagggcaaaattatc

SEQ ID NO: 71 - RNA, 21 nt, Synthetic construct
  source 1..21: mol_type = other RNA
tatccaagggcaaaattatcc

SEQ ID NO: 72 - RNA, 21 nt, Synthetic construct
  source 1..21: mol_type = other RNA
gggcaaaattatccactttgg

SEQ ID NO: 73 - RNA, 21 nt, Synthetic construct
  source 1..21: mol_type = other RNA
ggcaaaattatccactttggc

SEQ ID NO: 74 - RNA, 21 nt, Synthetic construct
  source 1..21: mol_type = other RNA
aattttcagatgcatcttatc

SEQ ID NO: 75 - RNA, 21 nt, Synthetic construct
  source 1..21: mol_type = other RNA
atcttatcaaagtataaacat

SEQ ID NO: 76 - RNA, 21 nt, Synthetic construct
  source 1..21: mol_type = other RNA
tcttatcaaagtataaacatt

SEQ ID NO: 77 - RNA, 21 nt, Synthetic construct
  source 1..21: mol_type = other RNA
cttatcaaagtataaacattc

SEQ ID NO: 78 - RNA, 21 nt, Synthetic construct
  source 1..21: mol_type = other RNA
tgattcagtctggttaaatat

SEQ ID NO: 79 - RNA, 21 nt, Synthetic construct
  source 1..21: mol_type = other RNA
gattcagtctggttaaatatt

SEQ ID NO: 80 - RNA, 21 nt, Synthetic construct
  source 1..21: mol_type = other RNA
ttaaatattgaagaaaaatgt

SEQ ID NO: 81 - RNA, 21 nt, Synthetic construct
  source 1..21: mol_type = other RNA
aactgtgtctcttaatatggc

SEQ ID NO: 82 - RNA, 21 nt, Synthetic construct
  source 1..21: mol_type = other RNA
ttggaaagagtatttcaattc

SEQ ID NO: 83 - RNA, 21 nt, Synthetic construct
  source 1..21: mol_type = other RNA
aaaagaagatagaagaaatag

SEQ ID NO: 84 - RNA, 21 nt, Synthetic construct
  source 1..21: mol_type = other RNA
aaatagctgctaaatataaac

SEQ ID NO: 85 - RNA, 21 nt, Synthetic construct
  source 1..21: mol_type = other RNA
gtgaagaaatgttgttacgat

SEQ ID NO: 86 - RNA, 21 nt, Synthetic construct
  source 1..21: mol_type = other RNA
tgaagaaatgttgttacgatg

SEQ ID NO: 87 - RNA, 21 nt, Synthetic construct
  source 1..21: mol_type = other RNA
ttcactgaatgttgtgtcgtc

SEQ ID NO: 88 - RNA, 21 nt, Synthetic construct
  source 1..21: mol_type = other RNA
gtgctaatatctctcataaag

SEQ ID NO: 89 - RNA, 21 nt, Synthetic construct
  source 1..21: mol_type = other RNA
aagaccctgttaccagtaagc

SEQ ID NO: 90 - RNA, 21 nt, Synthetic construct
  source 1..21: mol_type = other RNA
gccagaaattcggagttattt

SEQ ID NO: 91 - RNA, 21 nt, Synthetic construct
  source 1..21: mol_type = other RNA
ccagaaattcggagttatttt

SEQ ID NO: 92 - RNA, 21 nt, Synthetic construct
  source 1..21: mol_type = other RNA
agaaattcggagttattttcc

SEQ ID NO: 93 - RNA, 21 nt, Synthetic construct
  source 1..21: mol_type = other RNA
aagaaaacagttgcagtttgc

SEQ ID NO: 94 - RNA, 21 nt, Synthetic construct
  source 1..21: mol_type = other RNA
tttcaaacactggtatatgtg

SEQ ID NO: 95 - RNA, 21 nt, Synthetic construct
  source 1..21: mol_type = other RNA
cttcctggaaatgaatatacc

SEQ ID NO: 96 - RNA, 21 nt, Synthetic construct
  source 1..21: mol_type = other RNA
aactgtttacaactataggac

SEQ ID NO: 97 - RNA, 21 nt, Synthetic construct
  source 1..21: mol_type = other RNA
actgtttacaactataggact

SEQ ID NO: 98 - RNA, 21 nt, Synthetic construct
  source 1..21: mol_type = other RNA
ctgtttacaactataggactt

SEQ ID NO: 99 - RNA, 21 nt, Synthetic construct
  source 1..21: mol_type = other RNA
aagcaagatatttttataata

SEQ ID NO: 100 - RNA, 25 nt, Synthetic construct
  source 1..25: mol_type = other RNA
tattataaaaatatcttgctttttt

SEQ ID NO: 101 - RNA, 23 nt, Synthetic construct
  source 1..23: mol_type = other RNA
gaatatttttggtgctgaaatga

SEQ ID NO: 102 - RNA, 23 nt, Synthetic construct
  source 1..23: mol_type = other RNA
cggaatatttttggtgctgaaat

SEQ ID NO: 103 - RNA, 23 nt, Synthetic construct
  source 1..23: mol_type = other RNA
acggaatatttttggtgctgaaa

SEQ ID NO: 104 - RNA, 23 nt, Synthetic construct
  source 1..23: mol_type = other RNA
ccataaacttgaatcacaatatt

SEQ ID NO: 105 - RNA, 23 nt, Synthetic construct
  source 1..23: mol_type = other RNA
gtatccataaacttgaatcacaa

SEQ ID NO: 106 - RNA, 23 nt, Synthetic construct
  source 1..23: mol_type = other RNA
gtgtatccataaacttgaatcac

SEQ ID NO: 107 - RNA, 23 nt, Synthetic construct
  source 1..23: mol_type = other RNA
gagattgttgcatcaaatgcttc

SEQ ID NO: 108 - RNA, 23 nt, Synthetic construct
  source 1..23: mol_type = other RNA
acttttaatagagattgttgcat

SEQ ID NO: 109 - RNA, 23 nt, Synthetic construct
  source 1..23: mol_type = other RNA
aacttttaatagagattgttgca

SEQ ID NO: 110 - RNA, 23 nt, Synthetic construct
  source 1..23: mol_type = other RNA
caggataacttttaatagagatt

SEQ ID NO: 111 - RNA, 23 nt, Synthetic construct
  source 1..23: mol_type = other RNA
aaattttttatcaggataacttt

SEQ ID NO: 112 - RNA, 23 nt, Synthetic construct
  source 1..23: mol_type = other RNA
atttattctctgaggataaatga

SEQ ID NO: 113 - RNA, 23 nt, Synthetic construct
  source 1..23: mol_type = other RNA
gaatttattctctgaggataaat

SEQ ID NO: 114 - RNA, 23 nt, Synthetic construct
  source 1..23: mol_type = other RNA
agagttttggaatttattctctg

SEQ ID NO: 115 - RNA, 23 nt, Synthetic construct
  source 1..23: mol_type = other RNA
gttttggttgtattgttaagatt

SEQ ID NO: 116 - RNA, 23 nt, Synthetic construct
  source 1..23: mol_type = other RNA
aaatacacataagaaactgggtt

SEQ ID NO: 117 - RNA, 23 nt, Synthetic construct
  source 1..23: mol_type = other RNA
gatacaacttccaaatacacata

SEQ ID NO: 118 - RNA, 23 nt, Synthetic construct
  source 1..23: mol_type = other RNA
gaaaaatgctttgatacaacttc

SEQ ID NO: 119 - RNA, 23 nt, Synthetic construct
  source 1..23: mol_type = other RNA
ggtttgtctgtatgaatgaagag

SEQ ID NO: 120 - RNA, 23 nt, Synthetic construct
  source 1..23: mol_type = other RNA
agtataaacaggtttgtctgtat

SEQ ID NO: 121 - RNA, 23 nt, Synthetic construct
  source 1..23: mol_type = other RNA
gagtataaacaggtttgtctgta

SEQ ID NO: 122 - RNA, 23 nt, Synthetic construct
  source 1..23: mol_type = other RNA
ggtctggagtataaacaggtttg

SEQ ID NO: 123 - RNA, 23 nt, Synthetic construct
  source 1..23: mol_type = other RNA
gtcattcaacgaataaactctaa

SEQ ID NO: 124 - RNA, 23 nt, Synthetic construct
  source 1..23: mol_type = other RNA
gatctatgaaagttaagacagtt

SEQ ID NO: 125 - RNA, 23 nt, Synthetic construct
  source 1..23: mol_type = other RNA
aggatctatgaaagttaagacag

SEQ ID NO: 126 - RNA, 23 nt, Synthetic construct
  source 1..23: mol_type = other RNA
agataattccaatatgatcaatt

SEQ ID NO: 127 - RNA, 23 nt, Synthetic construct
  source 1..23: mol_type = other RNA
gagataattccaatatgatcaat

SEQ ID NO: 128 - RNA, 23 nt, Synthetic construct
  source 1..23: mol_type = other RNA
aaagagataattccaatatgatc

SEQ ID NO: 129 - RNA, 23 nt, Synthetic construct
  source 1..23: mol_type = other RNA
ggaatcttgaagtcaggaaaaga

SEQ ID NO: 130 - RNA, 23 nt, Synthetic construct
  source 1..23: mol_type = other RNA
gattagacggaatcttgaagtca

SEQ ID NO: 131 - RNA, 23 nt, Synthetic construct
  source 1..23: mol_type = other RNA
ggattagacggaatcttgaagtc

SEQ ID NO: 132 - RNA, 23 nt, Synthetic construct
  source 1..23: mol_type = other RNA
catatctaggattagacggaatc

SEQ ID NO: 133 - RNA, 23 nt, Synthetic construct
  source 1..23: mol_type = other RNA
cacataccatatctaggattaga

SEQ ID NO: 134 - RNA, 23 nt, Synthetic construct
  source 1..23: mol_type = other RNA
gaaaagtcctctttatatttagc

SEQ ID NO: 135 - RNA, 23 nt, Synthetic construct
  source 1..23: mol_type = other RNA
atatcttgcttttatagtaattt

SEQ ID NO: 136 - RNA, 23 nt, Synthetic construct
  source 1..23: mol_type = other RNA
tattataaaaatatcttgctttt

SEQ ID NO: 137 - RNA, 23 nt, Synthetic construct
  source 1..23: mol_type = other RNA
agtgactactttattataaaaat

SEQ ID NO: 138 - RNA, 23 nt, Synthetic construct
  source 1..23: mol_type = other RNA
atataaacgtcagcctcagtgac

SEQ ID NO: 139 - RNA, 23 nt, Synthetic construct
  source 1..23: mol_type = other RNA
gatataaacgtcagcctcagtga

SEQ ID NO: 140 - RNA, 23 nt, Synthetic construct
  source 1..23: mol_type = other RNA
catttctttttgatcatctttta

SEQ ID NO: 141 - RNA, 23 nt, Synthetic construct
  source 1..23: mol_type = other RNA
catttatcaacattgtgttttgc

SEQ ID NO: 142 - RNA, 23 nt, Synthetic construct
  source 1..23: mol_type = other RNA
ccatttatcaacattgtgttttg

SEQ ID NO: 143 - RNA, 23 nt, Synthetic construct
  source 1..23: mol_type = other RNA
cttctaaactgtagtatgacagt

SEQ ID NO: 144 - RNA, 23 nt, Synthetic construct
  source 1..23: mol_type = other RNA
ggtacttgttgtttaaatcttct

SEQ ID NO: 145 - RNA, 23 nt, Synthetic construct
  source 1..23: mol_type = other RNA
aaggtacttgttgtttaaatctt

SEQ ID NO: 146 - RNA, 23 nt, Synthetic construct
  source 1..23: mol_type = other RNA
atataaaggtacttgttgtttaa

SEQ ID NO: 147 - RNA, 23 nt, Synthetic construct
  source 1..23: mol_type = other RNA
aatataaaggtacttgttgttta

SEQ ID NO: 148 - RNA, 23 nt, Synthetic construct
  source 1..23: mol_type = other RNA
caatataaaggtacttgttgttt

SEQ ID NO: 149 - RNA, 23 nt, Synthetic construct
  source 1..23: mol_type = other RNA
gcaatataaaggtacttgttgtt

SEQ ID NO: 150 - RNA, 23 nt, Synthetic construct
  source 1..23: mol_type = other RNA
gactgttacagcaatataaaggt

SEQ ID NO: 151 - RNA, 23 nt, Synthetic construct
  source 1..23: mol_type = other RNA
atttgatgccaggtatttctgcc

SEQ ID NO: 152 - RNA, 23 nt, Synthetic construct
  source 1..23: mol_type = other RNA
gtcaagcgaatctttaacctgca

SEQ ID NO: 153 - RNA, 23 nt, Synthetic construct
  source 1..23: mol_type = other RNA
ggtcaagcgaatctttaacctgc

SEQ ID NO: 154 - RNA, 23 nt, Synthetic construct
  source 1..23: mol_type = other RNA
gacattaaactccagcaccgtca

SEQ ID NO: 155 - RNA, 23 nt, Synthetic construct
  source 1..23: mol_type = other RNA
agttttgacattaaactccagca

SEQ ID NO: 156 - RNA, 23 nt, Synthetic construct
  source 1..23: mol_type = other RNA
cagttttgacattaaactccagc

SEQ ID NO: 157 - RNA, 23 nt, Synthetic construct
  source 1..23: mol_type = other RNA
ctattgctcggtaaccttccctg

SEQ ID NO: 158 - RNA, 23 nt, Synthetic construct
  source 1..23: mol_type = other RNA
gctattgctcggtaaccttccct

SEQ ID NO: 159 - RNA, 23 nt, Synthetic construct
  source 1..23: mol_type = other RNA
gatgagtatgctattgctcggta

SEQ ID NO: 160 - RNA, 23 nt, Synthetic construct
  source 1..23: mol_type = other RNA
ggttatcagtccaatcaatataa

SEQ ID NO: 161 - RNA, 23 nt, Synthetic construct
  source 1..23: mol_type = other RNA
gcttttgggggtaacaataatat

SEQ ID NO: 162 - RNA, 23 nt, Synthetic construct
  source 1..23: mol_type = other RNA
gtcaatatatgggcttttggggg

SEQ ID NO: 163 - RNA, 23 nt, Synthetic construct
  source 1..23: mol_type = other RNA
agttattttgtcaatatatgggc

SEQ ID NO: 164 - RNA, 23 nt, Synthetic construct
  source 1..23: mol_type = other RNA
gagttattttgtcaatatatggg

SEQ ID NO: 165 - RNA, 23 nt, Synthetic construct
  source 1..23: mol_type = other RNA
attatagtgagttattttgtcaa

SEQ ID NO: 166 - RNA, 23 nt, Synthetic construct
  source 1..23: mol_type = other RNA
aattatagtgagttattttgtca

SEQ ID NO: 167 - RNA, 23 nt, Synthetic construct
  source 1..23: mol_type = other RNA
taattatagtgagttattttgtc

SEQ ID NO: 168 - RNA, 23 nt, Synthetic construct
  source 1..23: mol_type = other RNA
atcaagtaattatagtgagttat

SEQ ID NO: 169 - RNA, 23 nt, Synthetic construct
  source 1..23: mol_type = other RNA
ataattttgcccttggataaaat

SEQ ID NO: 170 - RNA, 23 nt, Synthetic construct
  source 1..23: mol_type = other RNA
gataattttgcccttggataaaa

SEQ ID NO: 171 - RNA, 23 nt, Synthetic construct
  source 1..23: mol_type = other RNA
ggataattttgcccttggataaa

SEQ ID NO: 172 - RNA, 23 nt, Synthetic construct
  source 1..23: mol_type = other RNA
ccaaagtggataattttgccctt

SEQ ID NO: 173 - RNA, 23 nt, Synthetic construct
  source 1..23: mol_type = other RNA
gccaaagtggataattttgccct

SEQ ID NO: 174 - RNA, 23 nt, Synthetic construct
  source 1..23: mol_type = other RNA
gataagatgcatctgaaaatttc

SEQ ID NO: 175 - RNA, 23 nt, Synthetic construct
  source 1..23: mol_type = other RNA
atgtttatactttgataagatgc

SEQ ID NO: 176 - RNA, 23 nt, Synthetic construct
  source 1..23: mol_type = other RNA
aatgtttatactttgataagatg

SEQ ID NO: 177 - RNA, 23 nt, Synthetic construct
  source 1..23: mol_type = other RNA
gaatgtttatactttgataagat

SEQ ID NO: 178 - RNA, 23 nt, Synthetic construct
  source 1..23: mol_type = other RNA
atatttaaccagactgaatcaga

SEQ ID NO: 179 - RNA, 23 nt, Synthetic construct
  source 1..23: mol_type = other RNA
aatatttaaccagactgaatcag

SEQ ID NO: 180 - RNA, 23 nt, Synthetic construct
  source 1..23: mol_type = other RNA
acatttttcttcaatatttaacc

SEQ ID NO: 181 - RNA, 23 nt, Synthetic construct
  source 1..23: mol_type = other RNA
gccatattaagagacacagtttg

SEQ ID NO: 182 - RNA, 23 nt, Synthetic construct
  source 1..23: mol_type = other RNA
gaattgaaatactctttccaagg

SEQ ID NO: 183 - RNA, 23 nt, Synthetic construct
  source 1..23: mol_type = other RNA
ctatttcttctatcttcttttgc

SEQ ID NO: 184 - RNA, 23 nt, Synthetic construct
  source 1..23: mol_type = other RNA
gtttatatttagcagctatttct

SEQ ID NO: 185 - RNA, 23 nt, Synthetic construct
  source 1..23: mol_type = other RNA
atcgtaacaacatttcttcacta

SEQ ID NO: 186 - RNA, 23 nt, Synthetic construct
  source 1..23: mol_type = other RNA
catcgtaacaacatttcttcact

SEQ ID NO: 187 - RNA, 23 nt, Synthetic construct
  source 1..23: mol_type = other RNA
gacgacacaacattcagtgaaag

SEQ ID NO: 188 - RNA, 23 nt, Synthetic construct
  source 1..23: mol_type = other RNA
ctttatgagagatattagcacgg

SEQ ID NO: 189 - RNA, 23 nt, Synthetic construct
  source 1..23: mol_type = other RNA
gcttactggtaacagggtcttca

SEQ ID NO: 190 - RNA, 23 nt, Synthetic construct
  source 1..23: mol_type = other RNA
aaataactccgaatttctggctt

SEQ ID NO: 191 - RNA, 23 nt, Synthetic construct
  source 1..23: mol_type = other RNA
aaaataactccgaatttctggct

SEQ ID NO: 192 - RNA, 23 nt, Synthetic construct
  source 1..23: mol_type = other RNA
ggaaaataactccgaatttctgg

SEQ ID NO: 193 - RNA, 23 nt, Synthetic construct
  source 1..23: mol_type = other RNA
gcaaactgcaactgttttcttct

SEQ ID NO: 194 - RNA, 23 nt, Synthetic construct
  source 1..23: mol_type = other RNA
cacatataccagtgtttgaaatg

SEQ ID NO: 195 - RNA, 23 nt, Synthetic construct
  source 1..23: mol_type = other RNA
ggtatattcatttccaggaagac

SEQ ID NO: 196 - RNA, 23 nt, Synthetic construct
  source 1..23: mol_type = other RNA
gtcctatagttgtaaacagttcc

SEQ ID NO: 197 - RNA, 23 nt, Synthetic construct
  source 1..23: mol_type = other RNA
agtcctatagttgtaaacagttc

SEQ ID NO: 198 - RNA, 23 nt, Synthetic construct
  source 1..23: mol_type = other RNA
aagtcctatagttgtaaacagtt

SEQ ID NO: 199 - DNA, 20 bp, Synthetic construct
  source 1..20: mol_type = other DNA
gatttggtcgtattgggcgc

SEQ ID NO: 200 - DNA, 20 bp, Synthetic construct
  source 1..20: mol_type = other DNA
actgaatgttgtgtcgtcgc

SEQ ID NO: 201 - DNA, 20 bp, Synthetic construct
  source 1..20: mol_type = other DNA
ctgaagcctgggattccata

SEQ ID NO: 202 - DNA, 20 bp, Synthetic construct
  source 1..20: mol_type = other DNA
cgagatccctccaaaatcaa

SEQ ID NO: 203 - DNA, 20 bp, Synthetic construct
  source 1..20: mol_type = other DNA
ttcccgttctcagccttgac

SEQ ID NO: 204 - DNA, 20 bp, Synthetic construct
  source 1..20: mol_type = other DNA
ccaacgccttgaatttccca

SEQ ID NO: 205 - DNA, 20 bp, Synthetic construct
  source 1..20: mol_type = other DNA
cgtcactccagatgggagat

SEQ ID NO: 206 - DNA, 20 bp, Synthetic construct
  source 1..20: mol_type = other DNA
tgacgatcttgaggctgttg

SEQ ID NO: 207 - RNA, 5480 nt, Homo sapiens
  source 1..5480: mol_type = mRNA
tatatccgtggtttcctgctacctccaaccatgggccttttgggaatactttgttttttaatcttcctggggaaaacctggggacaggagcaaacatatgtcatttcagcaccaaaaatattccgtgttggagcatctgaaaatattgtgattcaagtttatggatacactgaagcatttgatgcaacaatctctattaaaagttatcctgataaaaaatttagttactcctcaggccatgttcatttatcctcagagaataaattccaaaactctgcaatcttaacaatacaaccaaaacaattgcctggaggacaaaacccagtttcttatgtgtatttggaagttgtatcaaagcatttttcaaaatcaaaaagaatgccaataacctatgacaatggatttctcttcattcatacagacaaacctgtttatactccagaccagtcagtaaaagttagagtttattcgttgaatgacgacttgaagccagccaaaagagaaactgtcttaactttcatagatcctgaaggatcagaagttgacatggtagaagaaattgatcatattggaattatctcttttcctgacttcaagattccgtctaatcctagatatggtatgtggacgatcaaggctaaatataaagaggacttttcaacaactggaaccgcatattttgaagttaaagaatatgtcttgccacatttttctgtctcaatcgagccagaatataatttcattggttacaagaactttaagaattttgaaattactataaaagcaagatatttttataataaagtagtcactgaggctgacgtttatatcacatttggaataagagaagacttaaaagatgatcaaaaagaaatgatgcaaacagcaatgcaaaacacaatgttgataaatggaattgctcaagtcacatttgattctgaaacagcagtcaaagaactgtcatactacagtttagaagatttaaacaacaagtacctttatattgctgtaacagtcatagagtctacaggtggattttctgaagaggcagaaatacctggcatcaaatatgtcctctctccctacaaactgaatttggttgctactcctcttttcctgaagcctgggattccatatcccatcaaggtgcaggttaaagattcgcttgaccagttggtaggaggagtcccagtaacactgaatgcacaaacaattgatgtaaaccaagagacatctgacttggatccaagcaaaagtgtaacacgtgttgatgatggagtagcttcctttgtgcttaatctcccatctggagtgacggtgctggagtttaatgtcaaaactgatgctccagatcttccagaagaaaatcaggccagggaaggttaccgagcaatagcatactcatctctcagccaaagttacctttatattgattggactgataaccataaggctttgctagtgggagaacatctgaatattattgttacccccaaaagcccatatattgacaaaataactcactataattacttgattttatccaagggcaaaattatccactttggcacgagggagaaattttcagatgcatcttatcaaagtataaacattccagtaacacagaacatggttccttcatcccgacttctggtctattacatcgtcacaggagaacagacagcagaattagtgtctgattcagtctggttaaatattgaagaaaaatgtggcaaccagctccaggttcatctgtctcctgatgcagatgcatattctccaggccaaactgtgtctcttaatatggcaactggaatggattcctgggtggcattagcagcagtggacagtgctgtgtatggagtccaaagaggagccaaaaagcccttggaaagagtatttcaattcttagagaagagtgatctgggctgtggggcaggtggtggcctcaacaatgccaatgtgttccacctagctggacttaccttcctcactaatgcaaatgcagatgactcccaagaaaatgatgaaccttgtaaagaaattctcaggccaagaagaacgctgcaaaagaagatagaagaaatagctgctaaatataaacattcagtagtgaagaaatgttgttacgatggagcctgcgttaataatgatgaaacctgtgagcagcgagctgcacggattagtttagggccaagatgcatcaaagctttcactgaatgttgtgtcgtcgcaagccagctccgtgctaatatctctcataaagacatgcaattgggaaggctacacatgaagaccctgttaccagtaagcaagccagaaattcggagttattttccagaaagctggttgtgggaagttcatcttgttcccagaagaaaacagttgcagtttgccctacctgattctctaaccacctgggaaattcaaggcgttggcatttcaaacactggtatatgtgttgctgatactgtcaaggcaaaggtgttcaaagatgtcttcctggaaatgaatataccatattctgttgtacgaggagaacagatccaattgaaaggaactgtttacaactataggacttctgggatgcagttctgtgttaaaatgtctgctgtggagggaatctgcacttcggaaagcccagtcattgatcatcagggcacaaagtcctccaaatgtgtgcgccagaaagtagagggctcctccagtcacttggtgacattcactgtgcttcctctggaaattggccttcacaacatcaatttttcactggagacttggtttggaaaagaaatcttagtaaaaacattacgagtggtgccagaaggtgtcaaaagggaaagctattctggtgttactttggatcctaggggtatttatggtaccattagcagacgaaaggagttcccatacaggatacccttagatttggtccccaaaacagaaatcaaaaggattttgagtgtaaaaggactgcttgtaggtgagatcttgtctgcagttctaagtcaggaaggcatcaatatcctaacccacctccccaaagggagtgcagaggcggagctgatgagcgttgtcccagtattctatgtttttcactacctggaaacaggaaatcattggaacatttttcattctgacccattaattgaaaagcagaaactgaagaaaaaattaaaagaagggatgttgagcattatgtcctacagaaatgctgactactcttacagtgtgtggaagggtggaagtgctagcacttggttaacagcttttgctttaagagtacttggacaagtaaataaatacgtagagcagaaccaaaattcaatttgtaattctttattgtggctagttgagaattatcaattagataatggatctttcaaggaaaattcacagtatcaaccaataaaattacagggtaccttgcctgttgaagcccgagagaacagcttatatcttacagcctttactgtgattggaattagaaaggctttcgatatatgccccctggtgaaaatcgacacagctctaattaaagctgacaactttctgcttgaaaatacactgccagcccagagcacctttacattggccatttctgcgtatgctctttccctgggagataaaactcacccacagtttcgttcaattgtttcagctttgaagagagaagctttggttaaaggtaatccacccatttatcgtttttggaaagacaatcttcagcataaagacagctctgtacctaacactggtacggcacgtatggtagaaacaactgcctatgctttactcaccagtctgaacttgaaagatataaattatgttaacccagtcatcaaatggctatcagaagagcagaggtatggaggtggcttttattcaacccaggacacaatcaatgccattgagggcctgacggaatattcactcctggttaaacaactccgcttgagtatggacatcgatgtttcttacaagcataaaggtgccttacataattataaaatgacagacaagaatttccttgggaggccagtagaggtgcttctcaatgatgacctcattgtcagtacaggatttggcagtggcttggctacagtacatgtaacaactgtagttcacaaaaccagtacctctgaggaagtttgcagcttttatttgaaaatcgatactcaggatattgaagcatcccactacagaggctacggaaactctgattacaaacgcatagtagcatgtgccagctacaagcccagcagggaagaatcatcatctggatcctctcatgcggtgatggacatctccttgcctactggaatcagtgcaaatgaagaagacttaaaagcccttgtggaaggggtggatcaactattcactgattaccaaatcaaagatggacatgttattctgcaactgaattcgattccctccagtgatttcctttgtgtacgattccggatatttgaactctttgaagttgggtttctcagtcctgccactttcacagtgtacgaataccacagaccagataaacagtgtaccatgttttatagcacttccaatatcaaaattcagaaagtctgtgaaggagccgcgtgcaagtgtgtagaagctgattgtgggcaaatgcaggaagaattggatctgacaatctctgcagagacaagaaaacaaacagcatgtaaaccagagattgcatatgcttataaagttagcatcacatccatcactgtagaaaatgtttttgtcaagtacaaggcaacccttctggatatctacaaaactggggaagctgttgctgagaaagactctgagattaccttcattaaaaaggtaacctgtactaacgctgagctggtaaaaggaagacagtacttaattatgggtaaagaagccctccagataaaatacaatttcagtttcaggtacatctaccctttagattccttgacctggattgaatactggcctagagacacaacatgttcatcgtgtcaagcatttttagctaatttagatgaatttgccgaagatatctttttaaatggatgctaaaattcctgaagttcagctgcatacagtttgcacttatggactcctgttgttgaagttcgtttttttgttttcttctttttttaaacattcatagctggtcttatttgtaaagctcactttacttagaattagtggcacttgcttttattagagaatgatttcaaatgctgtaactttctgaaataacatggccttggagggcatgaagacagatactcctccaaggttattggacaccggaaacaataaattggaacacctcctcaaacctaccactcaggaatgtttgctggggccgaaagaacagtccattgaaagggagtattacaaaaacatggcctttgcttgaaagaaaataccaaggaacaggaaactgatcattaaagcctgagtttgctttcaaaaaaaaaaaaaaaaaa

SEQ ID NO: 208 - RNA, 5384 nt, Macaca mulatta
  source 1..5384: mol_type = mRNA
catgatttcctgctacctccaaccatgggccttttgggaatactttgttttttaatcttcctgggaaaaacttggggacaggagcaaacatatgtcatttcagcaccaaaaatattccgtgttggagcatctgaaaacattgtgattcaagtttatggatacactgaagcatttgatgcaacaatctctattaaaagttatcctgataaaaaatttagttactcctcaggccatgttcatttatcctcagagaataaattccaaaactcggcagtcttaacaatacaaccaaaacaattacctggaggacaaaaccaagtttcttatgtgtatttggaagttgtatcaaagcatttttcaaaatcaaaaaaaattccaataacctatgacaatggatttctcttcattcatacagacaaacctgtttatactccagaccaatcagtaaaggttagagtttattcgttgaatgatgacttgaagccagccaaaagagaaactgtcttaactttcatagatcctgaaggatcagaaattgacatggtagaagaaattgatcatattggaattatctcttttcctgacttcaagattccgtctaatcctagatatggtatgtggatgatccaggctaaatataaagaggacttttcaacaactggaactgcattttttgaagttaaagaatatgtcttgccacatttttctgtctcagtagaaccagaaagtaatttcattggttataagaactttaagaattttgaaattactataaaagcaagatatttttataataaagtagtcactgaggctgatgtttatatcacatttggaataagagaagacttaaaagatgatcaaaaagaaatgatgcaaacagcaatgcaaaacacaatgttgataaatggaattgctcaagtcacatttgattctgaaacagcagtcaaagaactgtcatactacagtttagaagatttaaacaacaagtacctttatattgctgtaacagtcatagagtctacaggtggattttctgaagaggcagaaatacctggcatcaaatatgtcctctctccctacaaactgaatttggttgctactcctcttttcctgaagcctgggattccatattccatcaaggtgcaggttaaagatgcgcttgaccagttggtaggaggggtcccagtaacactgaatgcacaaacaattgatgtcaaccaagagacatctgacttggagccaaggaaaagtgtaacacgtgttgatgatggagtagcttcgtttgtggttaatctcccatctggagtgacggtgctggagtttaatgtcaaaactgatgctccagatcttccagacgaaaatcaggccagggaaggttaccgagcaatagcatactcatctctcagccaaagttacctttatatcgattggactgataaccacaaggctttgctagtgggagaatatttgaatattattgttacccccaaaagcccatatattgacaaaataactcactataattacttgattttatccaagggcaaaattatccactttggcacaagggagaaactttcagatgcatcttatcaaagtataaacattccagtaacgcagaacatggttccttcatcccgactcctggtctattacatcgtcacaggagagcagacagcagaattagtgtctgattcagtctggttaaatattgaagaaaaatgtggcaaccagctccaggttcatctgtctcctgatgcagatacatattctccaggccaaactgtgtctcttaatatggtaactgggatggattcctgggtggcattaacagcagtggacagcgctgtgtatggagtccaaagaagagccaaaaagcccttggaaagagtatttcaattcttagagaagagtgatctgggctgtggggcaggtggtggcctcaacaatgccaatgtgttccacctagctggacttaccttcctcactaatgcaaatgcagatgactcccaagaaaatgatgaaccttgtaaagaaattatcaggccaagaagaatgctacaagagaagatagaagaaatagctgctaaatataaacatttagtagtgaagaaatgttgttacgatggagtccgtattaatcatgatgaaacctgtgagcagcgagctgcacggattagtgtagggccgagatgcgtcaaagctttcactgaatgttgtgtcgtcgcaagccagctccgtgctaataactctcataaagacttgcaattgggaaggctacacatgaagaccctgttaccagtaagcaagccagaaattcggagttattttccagaaagctggttatgggaagttcatcttgttcccagaagaaaacagttgcagtttgccctacctgattctgtaactacctgggaaattcaaggtgttggcatttcaaacagtggtatatgtgttgctgatactattaaggcaaaggtgttcaaagatgtcttcctggaaatgaatataccatattctgttgtacgaggagaacaggtccagttgaaaggaactgtttacaactataggacttctgggatgcagttctgtgttaaaatgtctgctgtggagggaatctgcacttcagaaagcccagtcattgatcatcagggcacaaagtcctccaaatgtgtgcgacagaaagtagagggctcctctaatcacttggtgacctttactgtgcttcctctggaaattggccttcagaacatcaatttctcactggagacttcgtttggaaaagaaatcttagtaaaatcgttacgagtggtgccagaaggtgtcaaaagggaaagctattctggtattactttggatcctaggggtatttatgnnnnnnnnnnnnnnnnnnnncgaaaggagttcccatacaggataccattagatttggtccccaaaacagaaatcaaaaggattttgagtgtaaaaggactgcttgtaggtgagatcttgtctgcagttctaagtcgggaaggcatcaatatcctaacccacctccccaaagggagtgcagaggcggagctgatgagcgttgtcccagtattctatgtttttcactacctggaaacaggaaatcattggaacatttttcattccgacccattaattgaaaagcggaacctggagaaaaaattaaaagaagggatggtgagcattatgtcctacagaaatgctgactattcttacagcgtgtggaagggtggcagtgctagcacttggttaacagcttttgctttaagagtacttggacaagtacataaatatgtagagcagaaccaaaattcaatatgtaattctttattgtggctggttgagaattatcagttagataatggatccttcaaggaaaattcacagtatcaaccaataaaattacagaaaatcaacacagctctaattaaagctgacacctttctgcttgaaaatacactgccagcccagagcacctttacattggccatttctgcctatgctctttccctgggagataaaactcacccacagttttgttcaattgtttcagctttgaagagagaagctttggttaaaggtaatccacccatttatcgtttttggaaagacagtcttcaacataaagacagctctgtacctaacactggtacagcacgtatggtagaaacaactgcctatgctttactcaccagtctgaacttgaaagacataaattatgttaacccaatcatcaaatggctatcagaagagcagaggtatggaggtggcttttattcaacccaggacacaatcaatgccatcgagggcctgacagaatattcactcctggttaaacagctccgcttgaatatggacatcgatgttgcttacaagcataaaggtcccttacataattataaaatgacagacaagaatttccttgggaggccagtagaggtgcttctcaatgatgacctcgttgtcagtacaggatttggcagtggcttggctacggtacatgtaacaactgtagttcacaaaaccagtacctctgaggaagtttgcagcttttatttgaaaattgatactcaggatattgaagcatcccactacagaggctacggaaactctgattacaaacgcatagtagcatgtgccagctacaagcccagcaaggaagaatcatcttctggatcctctcatgcagtgatggacatctccttgcctactggaatcaatgcaaatgaagaagacttaaaagctcttgtggaaggggtggatcagctattcactgattaccaaataaaagatggacatgttattctgcaactgaattcgatcccctccagtgatttcctttgtgtacgattccggatttttgaactctttgaagttgggtttcttagtcctgccactttcacagtgtatgaataccacagaccagataaacagtgtaccatgttttatagcacttccaatatcaaaattcagaaagtctgtgaaggagccacgtgcaagtgtatagaagctgattgtgggcaaatgcagaaagaattggatctgacaatctctgcagagactagaaaacaaacagcatgtaacccagagattgcatatgcttataaagttatcatcacatccatcactacagaaaatgtttttgtcaagtacaaggcaacccttctggatatctacaaaactggggaagctgttgctgaaaaagactctgaaatcaccttcattaaaaaggtaacctgcactaacgctgagctggtgaaaggaagacagtacttaattatggggaaagaagctctccagataaaatacaatttcactttcaggtacatctaccctttagattccttgacctggattgaatactggcctagagacacaacatgttcatcgtgtcaagcatttttagctaatttagatgaatttgctgaagacatctttttaaatggatgctaaaattcctgaagttcagctgcatacagtttgcacttatggactcctgttgttgaagtttgtttttttttctcgtttttttgtctttaaacattcacagctggtcttatttgtaaagctcactttacttagaattagtggcacttgcttttattagagaatgattttaaacgctgtaactttctgaaataacatggccttggagggcatgaagacagatactcctccaaggttattggacaccggaaacaataaattagaacacctcctcaaacctaccacttaggaatgtttgctggagccgaaagaacagtccattgaaatggagtattacaaaaacatggcctttgcttgaaagaaaataccaggggacaggaaactgatcattaaagcctgagtttgctttcaaactgtgctaaaaa

SEQ ID NO: 209 - RNA, 5448 nt, Mus musculus
  source 1..5448: mol_type = mRNA
tttaaaaggaaagtggttacagggaggccatgcccatgggtttatgccgctaccagccatgggtctttggggaatactttgtcttttaattttcctggacaaaacttggggacaggaacaaacctacgtcatttcagcacccaaaatcctccgggtcggctcgtctgaaaatgtggtaattcaagtccatggctacactgaagcatttgatgcaactctttctctaaaaagctatcctgacaaaaaagtcaccttctcttcaggctatgttaatttgtccccggaaaacaaattccaaaacgcggcactgttgacactacagcccaatcaagttcctagagaagaaagcccagtctctcacgtgtatctggaagttgtgtcaaaacacttttcaaaatcaaagaaaataccaattacctataacaatggaattctcttcatccatacagacaaacctgtttacacgccggaccagtcagtaaagatcagagtctattctctgggtgacgacttgaagccagccaaacgggagactgtcttaactttcatagaccccgaaggatcagaagttgacattgtagaagaaaatgattacaccggaattatctcttttcctgacttcaagattccatctaatcccaagtatggtgtttggacaattaaagctaactataagaaggattttacaacaactggaactgcatactttgaaattaaagaatatgtcttgccacgattctctgtttcaatagaactagaaagaaccttcattggctataaaaactttaagaactttgaaatcactgtgaaagcaagatatttttataataaagtggtacctgatgctgaagtgtatgccttttttggattgagagaggacataaaagatgaggagaagcagatgatgcacaaagccacacaagccgcaaagttggttgacggagttgctcagatctcttttgattctgaaacagcagttaaagagctgtcctacaacagtctagaagacttaaacaacaagtacctttatattgcagtaacagtcacagaatcttcaggtggattttcagaagaggcagaaatccctggagtcaaatatgtcctctctccctacacactgaatttggtcgctactcctcttttcgtgaagcccgggattccattttccatcaaggcacaggttaaagattcactcgagcaggcggtaggaggggtcccagtaactctgatggcacaaacagtcgatgtgaatcaagagacatctgacttggaaacaaagaggagcatcactcatgacactgatggagtagctgtgtttgtgctgaacctcccatcaaatgtgacggtgctaaagtttgagatcagaactgatgacccagaacttcccgaagaaaatcaagccagcaaagagtacgaagcagttgcgtactcgtctctcagccaaagttacatttacatcgcttggactgaaaactacaagcccatgcttgtgggagaatacctgaatattatggttacccccaagagcccatatatcgacaaaataactcactataattacttgattttatccaaaggcaaaattgtacagtacggcacaagagagaaacttttctcctcaacttatcaaaatataaatattccagtgacacagaacatggttccttcagcacgactcctggtctattacatagtcacaggggagcaaacagcagaattagtggctgacgcagtctggataaatattgaggagaagtgtggcaaccagctccaggtccatctgtctccagatgaatatgtgtattctccaggccaaactgtgtcccttgacatggtgactgaagcagactcatgggtagcactatcagcagtggacagagctgtgtataaagtccagggaaacgccaaaagggccatgcaaagagtctttcaagctttggatgaaaagagtgacctgggctgtggggcaggtggtggccatgacaatgcagatgtattccatctagctgggctcaccttcctcaccaacgcaaacgcagatgactcccattatcgtgatgactcttgtaaagaaattctcaggtcaaagagaaacctgcatctcctaaggcagaaaatagaagaacaagctgctaagtacaaacatagtgtgccaaagaaatgctgctatgacggagcccgagtgaacttctacgaaacctgtgaggagcgagtggcccgggttaccataggccctctctgcatcagggccttcaacgagtgctgtactattgcgaacaagatccgaaaagaaagcccccataaacctgtccaactgggaaggatccacattaagaccctgttaccagtgatgaaggcagatatccgaagctactttccagagagctggctatgggaaattcatcgcgttcccaaaagaaaacagctgcaggtcacgctgcctgactcactaacgacttgggaaattcaaggcattggcatttcagacaatggtatatgtgttgctgatacactcaaggcaaaggtgttcaaagaagtcttcctggagatgaacataccatattctgttgtgcgaggagaacagatccaattgaaaggaactgtttacaactatatgacctcagggacaaagttctgtgttaaaatgtctgctgtggaggggatctgcacttcaggaagctcagctgctagccttcacacctccaggccctccagatgtgtgttccagaggatagagggctcgtccagtcacttggtgaccttcaccctgcttcctctggaaattggccttcactccataaacttctcactagagacctcatttgggaaagacatcttagtaaagacattacgggtagtgccagaaggagtcaagagggaaagctatgccggcgtgattctggaccctaagggaattcgtggtattgttaacagacgaaaggaattcccatacaggatcccattagatttggtccccaagaccaaagttgaaaggattttgagtgtcaaaggactgcttgtaggggagttcttgtccacggttctgagtaaggaaggcatcaacatcctaacccacctccccaagggcagtgcagaggcagagctcatgagcatagctccggtgttctatgttttccactacctggaagcaggaaaccattggaatattttctatcctgatacactgagtaaaagacagagcctggagaaaaaaataaaacaaggggtggtgagcgtcatgtcctacagaaacgctgactattcctacagcatgtggaagggggcgagcgctagtacctggctgacagcttttgctctgagagtgcttggacaggtggccaagtatgtaaaacaggatgaaaactcaatttgtaactctttgctatggctggttgagaagtgtcagctggaaaacggctctttcaaggaaaattcccaatatctaccaataaaattacagggtactttgcctgctgaagcccaagagaaaactttgtatcttacagccttttctgtgattggaattagaaaggcagttgacatatgccccaccatgaaaatccacacagcgctagataaagccgactccttcctgcttgaaaacaccctgccatccaagagcaccttcacactggccattgtagcctatgctctttccctaggagacagaacccacccgaggtttcgtctaattgtgtcggccctgaggaaggaagcttttgttaaaggtgatccgcccatttaccgttactggagagataccctcaaacgtccagacagctctgtgcccagcagcggcacagcaggtatggttgaaaccacagcctatgctttgctcgccagcctgaaactgaaggatatgaattacgccaaccccatcatcaagtggctatctgaagagcagaggtatggaggcggcttttattccacccaggatacgattaatgccatcgagggcctgacagaatattcactcctgttaaaacaaattcatttggatatggacatcaatgtcgcctacaaacacgaaggtgacttccacaagtataaggtgacagagaagcatttcctggggaggccagtggaggtatctctcaatgatgaccttgttgtcagcacaggctacagcagtggcttggccacagtatatgtaaaaactgtggttcacaaaattagtgtctctgaggaattttgcagcttttacttgaaaattgatacccaagatattgaagcatccagccacttcaggctcagtgactctggattcaagcgcataatagcatgtgccagctacaagcccagcaaggaggagtcaacatccgggtcctcccatgcagtaatggatatatcactgccgactggaatcggagcaaacgaggaagatttacgggctcttgtggaaggagtggatcaactactaactgattaccagatcaaagatggccatgtcattctgcaactgaattcgatcccctccagagatttcctctgtgtccggttccggatatttgaacttttccaagttgggtttctgaatcctgctaccttcacggtgtacgagtatcacagaccagataagcagtgcaccatgatttatagcatttctgacaccaggcttcagaaagtctgtgaaggagcagcttgcacatgtgtggaagctgactgtgcgcaactgcaggcagaagtagacctagccatctctgcagactccagaaaagagaaagcctgtaaaccagagactgcatatgcttataaagtcaggatcacatcagccactgaagaaaatgtttttgtcaagtacactgcgactcttctggtcacttacaaaacaggggaagctgctgatgagaattcggaggtcaccttcattaaaaagatgagctgtaccaatgccaacctggtgaaagggaagcagtatttaatcatgggcaaagaggttctgcagatcaaacacaatttcagtttcaagtatatataccctctagattcctccacctggattgaatattggcccacagacacaacgtgtccatcctgtcaagcatttgtagagaatttgaataactttgctgaagacctctttttaaacagctgtgaatgaaaagttctgctgcacgaagattcctcctgcggcggggggattgctcctcctctggcttggaaacctagcctagaatcagatacactttctttagagtaaagcacaagctgatgagttacgactttgtgaaatggatagccttgaggggaggcgaaaacaggtcccccaaggctatcagatgtcagtgccaatagactgaaacaagtctgtaaagttagcagtcaggggtgttggttggggccggaagaagagacccactgaaactgtagccccttatcaaaacatatccttgcttgaaagaaaaataccaaggacagaaaatgccataaaatcttgactttgcactc

SEQ ID NO: 210 - RNA, 4516 nt, Rattus norvegicus
  source 1..4516: mol_type = mRNA
atgaagacaggaatgggtcaggggatggatagcacagagaccgacagatgtcctacagcccgccatcatctttccggaaacattaactcagtgcttgctgcccttgtaggtgggttttcggaagaggcagaaattcctggcatcaaatacgtcctctctccctatacactgaatttggtcgctacccctcttttcctgaagcctgggattccattttccatcaaggtacaggttaaggattcactcgagcagttggtaggaggggtcccagtaactctgatggcacaaacagtcaatgtgaatcaagagacatctgacttggaaccaaagaggagcatcacacactctgctgatggagtggcttcatttgtggtgaacctcccatcagaagtgacatcactgaagtttgaggtcaaaactgatgccccggaacttcccgaagaaaatcaagccagcaaagaatatgaagcagttacatactcatccctcagccagagttacatttacattggctggactgaaaactacaagcccatgcttgtgggagaatatctgaatattatcgtcacccccaagagtccatatattgacaaaataactcactataattacttgattttatccaaaggcaaaattgtacagtatggcacaaaggagaaacttctctattcatcttatcaaaatataaacatcccagtgacacaggacatggttccttcagcgcggctcctggtctattacatagtcacgggggagcagacagcagaattggtggctgacgcagtctggataaacattgaggagaagtgtggcaaccagctccaggtccatctgtctccagataaagacgtgtattctccaggccaaactgtgtcccttgacatggtgactgaagcagactcatgggtggcactatctgcggtggacagcgctgtgtatggagtccggggaaaagccaaaagggccatgcaaagagtgttccaagcttttgatgacaagagtgacctgggctgtggggcaggtggtggccgtgacaatgtagatgtattccatctagctgggctcaccttcctcaccaatgcaaacgcagatgactcccaataccacgatgactcttgtaaggaaattctcaggccaaagagagacctgcagctcctgcatcagaaagtggaagaacaagctgctaaatacaaacaccgtgtgcccaagaaatgctgttatgatggagcccgagaaaacaaatacgaaacctgtgagcagcgagttgcccgggtgaccataggcccacactgcatcagggccttcaacgagtgttgtactattgcggataagatccgaaaagaaagccaccacaaaggcatgctgttgggaaggatccaaataaaggccctgttaccagtgatgaaggcagaaatccgaagctactttccagagagctggctatgggaagttcatcgtgttcccaaaagaaaccagctgcaggttgcactgcctgactcactgacgacctgggaaattcaaggcatcggcatctcagacaatggtatatgtgttgctgacacactcaaggcaaaggtgttcaaagatgtcttcctggagatgaacataccatattctgttgtacgaggggagcagatccaattgaagggaaccgtttacaattataggacctctgggacaatgttctgtgttaaaatgtctgccgtggagggaatctgcactccaggaagctcggctgctagccctcagacctctaggtcctccagatgtgtgcgccagagaatagagggctcctccagtcacttggtgaccttcagcctgcttcctctggaaattggccttcactccataaacttctcactagagacttcatttgggaaagaaatcttagtgaagacattacgggtagtgccagaagggatcaaaagggaaagctatgctggtgtgactctggaccccaggggagtttatggtattgttaacagacgaaaggaattcccatacaggataccattagatttggtccccaaaaccaacgtcaaaaggattttgagtgtaaaaggactgcttataggggaattcttgtccacggttctgagtaaagaaggcatcgacatcctaacccacctccccaagggcagcgccgaggcagaactcatgagcatagtcccggtgttctacgttttccactacctggaagcaggaaaccattggaatattttccaccctgatacgttagctagaaaacagagcctgcagaaaaaaataaaagaagggctggtgagcgtcatgtcctacagaaacgctgactattcctacagcatgtggaagggagcaagctctagtgcctggctgacagcttttgctctgagagtgcttggacaggtgaacaagtatgtgaaacaagaccaatactcgatctgtaactccttgttatggctgattgagaagtgtcagctggaaaacggatctttcaaggaaaattcccaatatctaccaataaaattacagggtactttgcctgctgaagcccaagagaacactttatatcttacagccttttctgtgattggaattagaaaggctattggcatatgccccacggagaaaatctacacagcgctggctaaagctgactccttcctacttgaaaggaccctgccttccaagagcaccttcaccctggccattgtggcctatgctctctccctgggagacagaacccacccgaagtttcgttctattgtgtcagccctgaagagggaagctttggttaaaggagacccgcccatttaccgtttctggagagacactctccaacgtccagacagctcagcacccaacagcggcacagcaggtatggtagaaaccacggcctatgctttgctcaccagcctgaacctgaaggagacgagttatgtcaacccgatcatcaagtggctatctgaggagcagaggtatggaggcggcttttattccacccaggataccattaacgccatcgagggcctgacagagtattcactcctggttaaacaacttcatttggatatggatatcaatgtctcctacaaacacaaaggggatttctaccagtataaagtgacagagaagaacttcctcgggaggccagtggaggtacccctcaatgatgacctcatcgtcaccacaggctatagcagtggcttggctacagtatatgtaaaaactgtggttcacaaaactagtgtcgctgaggaattttgcagcttttacttgaaaattgatacccaagaagttgaagcctccagctacctcagctacagtgactcgggacacaagcgcataatagcctgtgccagctacaagcccagcaaggaggagtcagcatctgggtcctcccatgcagtaatggatatactgctgccgaccggaatcggagcaaaccaagaagatttacgagctcttgtggaaggagtagatcaactcctaactgattaccagatcaaagacagtcatgttattctgcaattgaattcgattccctccagagatttcctttgtgttcggttccggatatttgaacttttccaagttgggtttctgaatcctgctacgttcacggtgtacgagtatcacagaccagataagcagtgtaccatgatttacagcacttctgacaccaaccttcagagagtctgtgaaggagcggcatgcaaatgcgttgaagctgattgtgggcaactgcaggcagaactggacctggccatctctgcagacaccaggaaagaaacagcatgtaaaccagagattgcatatgcttataaggtcaggatcacgtcggccacggaagaaaacatttttgtcaagtacactgcgacgcttctggatatttacaaaacaggggaagccgctgctgagaaggactctgagatcaccttcattaaaaagataagctgtaccaacgccaacctggtgaaaggaaagcaatatttaatcatgggcaaagaggctctgcagatcaaacacaatttcagtttcaagtatatataccctctagattcctccacctggattgaatattggcccacagacacaacgtgtccatcctgccaagcgtttgtagctaatttggacgagttcgctgaagacatctttctaaatggctgtgaaaatgcctgaggaagttctgctgcgtggccttcccgggtactcctgttggtggctcctaggagccaggatcgcttggaaacttagcctagaatcggatacattttctttatagtaaagcgtaagttgaagagttactttgtgaaacaaaatagccttgtggagagccgaaggcaggtcccccaaggctattggacatcagcaccaataagctggaacaagtctgtaacgttagcagccaggggtgtttgttggggccggaagaagagactcactgaaattgtagccccttaggaaaacatggtcttgcttgaaaaaaaaaataccaaggacagaaaatgccataaaagcttgactttgcactcaa

SEQ ID NO: 211 - RNA, 5464 nt, Homo sapiens
  source 1..5464: mol_type = mRNA
atatccgtggtttcctgctacctccaaccatgggccttttgggaatactttgttttttaatcttcctggggaaaacctggggacaggagcaaacatatgtcatttcagcaccaaaaatattccgtgttggagcatctgaaaatattgtgattcaagtttatggatacactgaagcatttgatgcaacaatctctattaaaagttatcctgataaaaaatttagttactcctcaggccatgttcatttatcctcagagaataaattccaaaactctgcaatcttaacaatacaaccaaaacaattgcctggaggacaaaacccagtttcttatgtgtatttggaagttgtatcaaagcatttttcaaaatcaaaaagaatgccaataacctatgacaatggatttctcttcattcatacagacaaacctgtttatactccagaccagtcagtaaaagttagagtttattcgttgaatgacgacttgaagccagccaaaagagaaactgtcttaactttcatagatcctgaaggatcagaagttgacatggtagaagaaattgatcatattggaattatctcttttcctgacttcaagattccgtctaatcctagatatggtatgtggacgatcaaggctaaatataaagaggacttttcaacaactggaaccgcatattttgaagttaaagaatatgtcttgccacatttttctgtctcaatcgagccagaatataatttcattggttacaagaactttaagaattttgaaattactataaaagcaagatatttttataataaagtagtcactgaggctgacgtttatatcacatttggaataagagaagacttaaaagatgatcaaaaagaaatgatgcaaacagcaatgcaaaacacaatgttgataaatggaattgctcaagtcacatttgattctgaaacagcagtcaaagaactgtcatactacagtttagaagatttaaacaacaagtacctttatattgctgtaacagtcatagagtctacaggtggattttctgaagaggcagaaatacctggcatcaaatatgtcctctctccctacaaactgaatttggttgctactcctcttttcctgaagcctgggattccatatcccatcaaggtgcaggttaaagattcgcttgaccagttggtaggaggagtcccagtaacactgaatgcacaaacaattgatgtaaaccaagagacatctgacttggatccaagcaaaagtgtaacacgtgttgatgatggagtagcttcctttgtgcttaatctcccatctggagtgacggtgctggagtttaatgtcaaaactgatgctccagatcttccagaagaaaatcaggccagggaaggttaccgagcaatagcatactcatctctcagccaaagttacctttatattgattggactgataaccataaggctttgctagtgggagaacatctgaatattattgttacccccaaaagcccatatattgacaaaataactcactataattacttgattttatccaagggcaaaattatccactttggcacgagggagaaattttcagatgcatcttatcaaagtataaacattccagtaacacagaacatggttccttcatcccgacttctggtctattacatcgtcacaggagaacagacagcagaattagtgtctgattcagtctggttaaatattgaagaaaaatgtggcaaccagctccaggttcatctgtctcctgatgcagatgcatattctccaggccaaactgtgtctcttaatatggcaactggaatggattcctgggtggcattagcagcagtggacagtgctgtgtatggagtccaaagaggagccaaaaagcccttggaaagagtatttcaattcttagagaagagtgatctgggctgtggggcaggtggtggcctcaacaatgccaatgtgttccacctagctggacttaccttcctcactaatgcaaatgcagatgactcccaagaaaatgatgaaccttgtaaagaaattctcaggccaagaagaacgctgcaaaagaagatagaagaaatagctgctaaatataaacattcagtagtgaagaaatgttgttacgatggagcctgcgttaataatgatgaaacctgtgagcagcgagctgcacggattagtttagggccaagatgcatcaaagctttcactgaatgttgtgtcgtcgcaagccagctccgtgctaatatctctcataaagacatgcaattgggaaggctacacatgaagaccctgttaccagtaagcaagccagaaattcggagttattttccagaaagctggttgtgggaagttcatcttgttcccagaagaaaacagttgcagtttgccctacctgattctctaaccacctgggaaattcaaggcgttggcatttcaaacactggtatatgtgttgctgatactgtcaaggcaaaggtgttcaaagatgtcttcctggaaatgaatataccatattctgttgtacgaggagaacagatccaattgaaaggaactgtttacaactataggacttctgggatgcagttctgtgttaaaatgtctgctgtggagggaatctgcacttcggaaagcccagtcattgatcatcagggcacaaagtcctccaaatgtgtgcgccagaaagtagagggctcctccagtcacttggtgacattcactgtgcttcctctggaaattggccttcacaacatcaatttttcactggagacttggtttggaaaagaaatcttagtaaaaacattacgagtggtgccagaaggtgtcaaaagggaaagctattctggtgttactttggatcctaggggtatttatggtaccattagcagacgaaaggagttcccatacaggatacccttagatttggtccccaaaacagaaatcaaaaggattttgagtgtaaaaggactgcttgtaggtgagatcttgtctgcagttctaagtcaggaaggcatcaatatcctaacccacctccccaaagggagtgcagaggcggagctgatgagcgttgtcccagtattctatgtttttcactacctggaaacaggaaatcattggaacatttttcattctgacccattaattgaaaagcagaaactgaagaaaaaattaaaagaagggatgttgagcattatgtcctacagaaatgctgactactcttacagtgtgtggaagggtggaagtgctagcacttggttaacagcttttgctttaagagtacttggacaagtaaataaatacgtagagcagaaccaaaattcaatttgtaattctttattgtggctagttgagaattatcaattagataatggatctttcaaggaaaattcacagtatcaaccaataaaattacagggtaccttgcctgttgaagcccgagagaacagcttatatcttacagcctttactgtgattggaattagaaaggctttcgatatatgccccctggtgaaaatcgacacagctctaattaaagctgacaactttctgcttgaaaatacactgccagcccagagcacctttacattggccatttctgcgtatgctctttccctgggagataaaactcacccacagtttcgttcaattgtttcagctttgaagagagaagctttggttaaaggtaatccacccatttatcgtttttggaaagacaatcttcagcataaagacagctctgtacctaacactggtacggcacgtatggtagaaacaactgcctatgctttactcaccagtctgaacttgaaagatataaattatgttaacccagtcatcaaatggctatcagaagagcagaggtatggaggtggcttttattcaacccaggacacaatcaatgccattgagggcctgacggaatattcactcctggttaaacaactccgcttgagtatggacatcgatgtttcttacaagcataaaggtgccttacataattataaaatgacagacaagaatttccttgggaggccagtagaggtgcttctcaatgatgacctcattgtcagtacaggatttggcagtggcttggctacagtacatgtaacaactgtagttcacaaaaccagtacctctgaggaagtttgcagcttttatttgaaaatcgatactcaggatattgaagcatcccactacagaggctacggaaactctgattacaaacgcatagtagcatgtgccagctacaagcccagcagggaagaatcatcatctggatcctctcatgcggtgatggacatctccttgcctactggaatcagtgcaaatgaagaagacttaaaagcccttgtggaaggggtggatcaactattcactgattaccaaatcaaagatggacatgttattctgcaactgaattcgattccctccagtgatttcctttgtgtacgattccggatatttgaactctttgaagttgggtttctcagtcctgccactttcacagtgtacgaataccacagaccagataaacagtgtaccatgttttatagcacttccaatatcaaaattcagaaagtctgtgaaggagccgcgtgcaagtgtgtagaagctgattgtgggcaaatgcaggaagaattggatctgacaatctctgcagagacaagaaaacaaacagcatgtaaaccagagattgcatatgcttataaagttagcatcacatccatcactgtagaaaatgtttttgtcaagtacaaggcaacccttctggatatctacaaaactggggaagctgttgctgagaaagactctgagattaccttcattaaaaaggtaacctgtactaacgctgagctggtaaaaggaagacagtacttaattatgggtaaagaagccctccagataaaatacaatttcagtttcaggtacatctaccctttagattccttgacctggattgaatactggcctagagacacaacatgttcatcgtgtcaagcatttttagctaatttagatgaatttgccgaagatatctttttaaatggatgctaaaattcctgaagttcagctgcatacagtttgcacttatggactcctgttgttgaagttcgtttttttgttttcttctttttttaaacattcatagctggtcttatttgtaaagctcactttacttagaattagtggcacttgcttttattagagaatgatttcaaatgctgtaactttctgaaataacatggccttggagggcatgaagacagatactcctccaaggttattggacaccggaaacaataaattggaacacctcctcaaacctaccactcaggaatgtttgctggggccgaaagaacagtccattgaaagggagtattacaaaaacatggcctttgcttgaaagaaaataccaaggaacaggaaactgatcattaaagcctgagtttgctttcaaa

SEQ ID NO: 212 - RNA, 5466 nt, Macaca fascicularis
  source 1..5466: mol_type = mRNA
atatccatgatttcctgctacctccaaccatgggccttttgggaatactttgttttttaatcttcctgggaaaaacttggggacaggagcaaacatatgtcatttcagcaccaaaaatattccgtgttggagcatctgaaaacattgtgattcaagtttatggatacactgaagcatttgatgcaacaatctctattaaaagttatcctgataaaaaatttagttactcctcaggccatgttcatttatcctcagagaataaattccaaaactcggcagtcttaacaatacaaccaaaacaattacctggaggacaaaaccaagtttcttatgtgtatttggaagttgtatcaaagcatttttcaaaatcaaaaaaaattccaataacctatgacaatggatttctcttcattcatacagacaaacctgtttatactccagaccaatcagtaaaggttagagtttattcgttgaatgatgacttgaagccagccaaaagagaaactgtcttaactttcatagatcctgaaggatcagaaattgacatggtagaagaaattgatcatattggaattatctcttttcctgacttcaagattccgtctaatcctagatatggtatgtggatgatccaggctaaatataaagaggacttttcaacaactggaactgcattttttgaagttaaagaatatgtcttgccacatttttctgtctcagtagaaccagaaagtaatttcattggttataagaactttaagaattttgaaattactataaaagcaagatatttttataataaagtagtcactgaggctgatgtttatatcacatttggaataagagaagacttaaaagatgatcaaaaagaaatgatgcaaacagcaatgcaaaacacaatgttgataaatggaattgctgaagtcacatttgattctgaaacagcagtcaaagaactgtcatactacagtttagaagatttaaacaacaagtacctttatattgctgtaacagtcatagagtctacaggtggattttctgaagaggcagaaatacctggcatcaaatatgtcctctctccctacaaactgaatttggttgctactcctcttttcctgaagcctgggattccatattccatcaaggtgcaggttaaagatgcgcttgaccagttggtaggaggggtcccagtaacactgaatgcacaaacaattgatgtcaaccaagagacatctgacttggagccaaggaaaagtgtaacacgtgttgatgatggagtagcttcgtttgtggttaatctcccatctggagtgacggtgctggagtttaatgtcaaaactgatgctccagatcttccagacgaaaatcaggccagggaaggttaccgagcaatagcatactcatctctcagccaaagttacctttatatcgattggactgataaccacaaggctttgctagtgggagaatatttgaatattattgttacccccaaaagcccatatattgacaaaataactcactataattacttgattttatccaagggcaaaattatccactttggcacaagggagaaactttcagatgcatcttatcaaagtataaacattccagtaacgcagaacatggttccttcatcccgactcttggtctattacatcgtcacaggagagcagacagcagaattagtgtctgattcagtctggttaaatattgaagaaaaatgtggcaaccagctccaggttcatctgtctcctgatgcagatacatattctccaggccaaactgtgtctcttaatatggtaactgggatggattcctgggtggcattaacagcagtggacagcgctgtgtatggagtccaaagaagagccaaaaagcccttggaaagagtatttcaattcttagagaagagtgatctgggctgtggggcaggtggtggcctcaacaatgccaatgtgttccacctagctggacttaccttcctcactaatgcaaatgcagatgactcccaagaaaatgatgaaccttgtaaagaaattatcaggccaagaagaatgctacaagagaagatagaagaaatagctgctaaatataaacatttagtagtgaagaaatgttgttacgatggagtccgtattaatcatgatgaaacctgtgagcagcgagctgcacggattagtgtagggccgagatgcgtcaaagctttcactgaatgttgtgtcgtcgcaagccagttccgtgctaataactctcataaagacttgcaattgggaaggctacacatgaagaccctgttaccagtaagcaagccagaaattcggagttattttccagaaagctggttatgggaagttcatcttgttcccagaagaaaacagttgcagtttgccctacctgattctgtaactacctgggaaattcaaggtgttggcatttcaaacagtggtatatgtgttgctgatactattaaggcaaaggtgttcaaagatgtcttcctggaaatgaatataccatattctgttgtacgaggagaacaggtccagttgaaaggaactgtttacaactataggacttctgggatgcagttctgtgttaaaatgtctgctgtggagggaatctgcacttcagaaagcccagtcattgatcatcagggcacaaagtcctccaaatgtgtgcgacagaaagtagagggctcctctaatcacttggtgacctttactgtgcttcctctggaaattggccttcagaacatcaatttctcactggagacttcgtttggaaaagaaatcttagtaaaatcgttacgagtggtgccagaaggtgtcaaaagggaaagctattctggtattactttggatcctaggggtatttatggtaccattagcagacgaaaggagttcccatacaggataccattagatttggtccccaaaacagaaatcaaaaggattttgagtgtaaaaggactgcttgtaggtgagatcttgtctgcagttctaagtcgggaaggcatcaatatcctaacccacctccccaaagggagtgcagaggcggagctgatgagcgttgtcccagtattctatgtttttcactacctggaaacaggaaatcattggaacatttttcattccgacccattaattgaaaagcggaacctggagaaaaaattaaaagaagggatggtgagcattatgtcctacagaaatgctgactattcttacagcgtgtggaagggtggcagtgctagcacttggttaacagcttttgctttaagagtacttggacaagtacataaatatgtagagcagaaccaaaattcaatatgtaattctttattgtggctggttgagaattatcagttagataatggatctttcaaggaaaattcacagtatcaaccaataaaattacagggtaccttgcctgttgaagcccgagagaacagcttatatcttacagcctttactgtgattggaattagaaaggcttttgatatatgccccctggtgaaaatcaacacagctctaattaaagctgacacctttctgcttgaaaatacactgccagcccagagcacctttacattggccatttctgcctatgctctttccctgggagataaaactcacccacagtttcgttcaattgtttcagctttgaagagagaagctttggttaaaggtaatccacccatttatcgtttttggaaagacagtcttcaacataaagacagctctgtacctaacactggtacagcacgtatggtagaaacaactgcctatgctttactcaccagtctgaacttgaaagacataaattatgttaacccaatcatcaaatggctatcagaagagcagaggtatggaggtggcttttattcaacccaggacacaatcaatgccatcgagggcctgacagaatattcactcctggttaaacagctccgcttgaatatggacatcgatgttgcttacaagcataaaggtcccttacataattataaaatgacagacaagaatttccttgggaggccagtagaggtgcttctcaatgatgacctcgttgtcagtacaggatttggcagtggcttggctacggtacatgtaacaactgtagttcacaaaaccagtacctctgaggaagtttgcagcttttatttgaaaattgatactcaggatattgaagcatcccactacagaggctacggaaactctgattacaaacgcatagtagcatgtgccagctacaagcccagcaaggaagaatcatcttctggatcctctcatgcagtaatggacatctccttgcctactggaatcaatgcaaatgaagaagacttaaaagctcttgtggaaggggtggatcagctattcactgattaccaaataaaagatggacatgttattctgcaactgaattcgatcccctccagtgatttcctttgtgtacgattccggatttttgaactctttgaagttgggtttcttagtcctgccactttcacagtgtatgaataccacagaccagataaacagtgtaccatgttttatagcacttccaatatcaaaattcagaaagtctgtgaaggagccacgtgcaagtgtatagaagctgattgtgggcaaatgcagaaagaattggatctgacaatctctgcagagactagaaaacaaacagcatgtaacccagagattgcatatgcttataaagttatcatcacatccatcactacagaaaatgtttttgtcaagtacaaggcaacccttctggatatctacaaaactggggaagctgttgctgagaaagactctgaaatcaccttcattaaaaaggtaacctgcactaacgctgagctggtgaaaggaagacagtacttaattatggggaaagaagctctccagataaaatacaatttcactttcaggtacatctaccctttagattccttgacctggattgaatactggcctagagacacaacatgttcatcgtgtcaagcatttttagctaatttagatgaatttgctgaagacatctttttaaatggatgctaaaattcctgaagttcagctgcatacagtttgcacttatggactcctgttgttgaagtttgttttttttctcgtttttttttctttaaacattcacagctggtcttatttgtaaagctcactttacttagaattagtggcacttgcttttattagagaatgattttaaacgctgtaactttctgaaataacatggccttggagggcatgaagacagatactcctccaaggttattggacaccggaaacaataaattagaacacctcctcaaacctaccacttaggaatgtttgctggagccgaaagaacagtccattgaaatggagtattacaaaaacatggcctttgcttgaaagaaaataccaggggacaggaaactgatcattaaagcctgagtttgctttcaaa